European Patent Application EP 4 772 647 A1, published July 8, 2026. Title: 抑制PCSK9基因表达的siRNA的制备方法. Applicant: 吉林凯莱英制药有限公司. The sequence listing filed with the application follows.

SEQUENCE LISTING (56 sequences)

SEQ ID NO: 1 - protein, 334 aa, Salmonellaenterica
MFKKYSSLENHYNSKFIEKLYSLGLTGGEWVAREKIHGTNFSLIIERDKVTCAKRTGPILPAEDFFGYEIILKNYADSIKAVQDIMETSAVVTYQVFGEFAGPGIQKNVDYGDKDFYVFDIIVTTESGDVTYVDDYMMESFCNTFKFKMAPLLGRGKFEELIKLPNDLDSVVQDYNFTVDHAGLVDANKCVWNAEAKGEVFTAEGYVLKPCYPSWLPNRNRVAIKCKNSKFSEKKKSDKPIKTKVELSEADNKLMGILACYVTLNRVNNVISKIGEIGPKDFGKVMGLTVQDILEETSREGITLTQADNPSLIKKELVKMVQDVLRPAWIELVS

SEQ ID NO: 2 - protein, 334 aa, YersiniaphagevB_YepM_ZN18
MFKKYSSLENHYNSKFIEKLYSLGLTGGEWVAREKIHGTNFSLIIERDKVTCAKRTGPILPAEDFFGYEIILKNYEDSIKAVQDIMETSAVVSYQVFGEFAGPGIQKNVDYGDKDFYVFDIIVTTESGDVTYVDDYMMESFCNTFKFKMAPLLGRGKFEELIKLPNDLDSVVQDYNFTVDHAGLVDANKCVWKAEAKGEVFTAEGYVLKPCYPSWLHNGNRVAIKCKNSKFSEKKKSDKPIKAKVELSEADNKLVGILACYVTLNRVNNVISKIGEIGPKDFGKVMGLTVQDILEETSREGITLTQADNPSLVKKELVKMVQDVLRPAWIELVS

SEQ ID NO: 3 - protein, 334 aa, Shigella phage pSs-1
MFKKYSSLENHYNSKFIEKLYSLGLTGGEWVAREKIHGTNFSLIIERDKVTCAKRTGPILPAEDFFGYEIILKNYADSIKAVQDIMETSAVVSYQVFGEFAGPGIQKNVDYGDKDFYVFDIIVTTESGDVTYVDDYMMESFCNTFKFKMAPLLGRGKFEELIKLPNDLDSVVQDYNFTVDHAGLVDANKCVWNAEAKCEVFTAEGYVLKPCYPSWLPNRNRVAIKCKNSKFSEKKKSDKPIKAKVELSEADNKLVGILACYVTLNRVNNVISKIGEIGPKDFGKVMGLTVQDILEETSREGITLTQADSPSLVKKELVKMVQDVLRPAWIELVS

SEQ ID NO: 4 - protein, 334 aa, Bacteriophage
MFKKYSSLENHYNSKFIEKLYSLGLTGGEWVAREKIHGTNFSLIIERDKVTCAKRTGPILPAEDFFGYEIILKNYADSIKAVQDIMETSAVVSYQVFGEFAGPGIQKNVDYCDKDFYVFDIIVTTESGDVTYVDDYMMESFCNTFKFKMAPLLGRGKFEELIKLPNDLDSVVQDYNFTVDHAGLVDANKCVWNAEAKGEVFTAEGYVLKPCYPSWLRNGNRVAIKCKNSKFSEKKKSDKPIKAKVELSEADNKLVGILACYVTLNRVNNVISKIGEIGPKDFGKVMGLTVQDILEETSREGITLTQADNPSLIKKELVKMVQDVLRPAWIELVS

SEQ ID NO: 5 - protein, 358 aa, Bacteriophage T7
MNIKTNPFKAVSFVESAIKKALDNAGYLIAEIKYDGVRGNICVDNTANSYWLSRVSKTIPALEHLNGFDVRWKRLLNDDRCFYKDGFMLDGELMVKGVDFNTGSGLLRTKWTDTKNQEFHEELFVEPIRKKDKVPFKLHTGHLHIKLYAILPLHIVESGEDCDVMTLLMQEHVKNMLPLLQEYFPEIEWQAAESYEVYDMVELQQLYEQKRAEGHEGLIVKDPMCIYKRGKKSGWWKMKPENEADGIIQGLVWGTKGLANEGKVIGFEVLLESGRLVNATNISRALMDEFTETVKEATLSQWGFFSPYGIGDNDACTINPYDGWACQISYMEETPDGSLRHPSFVMFRGTEDNPQEKM

SEQ ID NO: 6 - protein, 335 aa, Bacteriophage dhaeg
MFKKYSSLENHYNSKFIEKLRTNGLTGGEWVAREKIHGTNFSLIIERDAVTCAKRTGPILPAEDFYGYEIVLKNYADSIKSIQDIMETSAAVSYQVFGEFAGTGIQKNVDYGDKDFYVFDIIVTTESGDVTYVDDYMMESFCKTFKFKMAPLLGRGKFEDLIKLPNDLDSVLPDYNFTVDNVGLAEANAHVWNAEAKGEVFTAEGYVLKPCYPLWLPNGNRVAIKCKNSKFSEKKKTDKPIKVAVVLSQDDLDLLQQFTDYVTVNRINNVISKIGEVSPKDFGKVMGLTVQDILEEAAREELELTDAENPVEVKKQLIECVKDTLRAVWIELVSK

SEQ ID NO: 7 - protein, 339 aa, Klebsiella phage KP27
MFKKYSSLTNHYEGKFINGVIMNGLTGGVWVAREKIHGANFSFITDDGITVTPAKRTDVVKPAEDFYGCSAVVAKYSPGIRKMWETLKKTGTYDDLVIQVYGEFAGRGVQKDVDYGEKDFYVFDIRVNGEFLPDNLCSLISRSHGLKMAPLLGYGTFEEIKELPITFESVVNKANSGIGSDNTVYGEFVYPIMDVEEGNIAEGFVMKPVSPAFMPNGERVAIKCKTTKFTEKKAKKATRFNAPVSLSEKDKNQLDEFVCYLTENRVKNVLSKLDLASITAKDFGRIMGLTVQDAIEEISRNHGPFLEQFEDPAMAKKLFVTEAQNMIRPVWGKILNHEF

SEQ ID NO: 8 - protein, 335 aa, Vibrio phage phi-ST2
MSFVKYTSLENSYRQAFVDKCDMLGVKEWVALEKIHGANFSFIVEFKPSTEEVPGEMSVTPAKRTSTIGANAMGDYDFYGCTSVVEAHIEKMQDISNWLFANDFIKNDETIIVYGELAGKGIQKEVNYGDKDFWAYDILCPETGEFLDWDVVLKACKFAGVKTTHEIARGTLDELLKIDPLFRSFHTPADVDSENVAEGFVVKQLKAEKRLHNGSRAILKVKNEKFKEKKNKQGKTPRAKVVLTEEQEKLHAAFSCYLTENRLRNVLSKIGKVEAKQFGMVSGLFVKDAKDEFERDERDEVAIPRDDWDVIKRSLVNVANEILRKNWLNIVDGTF

SEQ ID NO: 9 - protein, 339 aa, Klebsiella phage KP15
MFKKYSSLTNHYEGKFINGVIMNGLTGGVWVAREKIHGANFSFITDDGITVTPAKRTDVVKPAEDFYGCSAVVAKYSPGIRKMWETLKKTGTYDDLVIQVYGEFAGRGVQKDVDYGEKDFYVFDIRVNGEFLPDNLCSLISRSHGLKMAPLLGYGTFEEIKELPITFESVVNKANSGIGSDNTVYGEFVYPIMDVEEGNIAEGFVMKPVSPAFMPNGERVAIKCKTTKFTEKKAKKATRFNAPVSLSEKDKNQLDEFVCYLTENRVKNVLSKLDLASITAKDFGRIMGLTVQDAIEEISRNHGPFIEQFEDPAMAKKLFVTEAQNMIRPVWGKILNHEF

SEQ ID NO: 10 - protein, 335 aa, Vibrio phage JN02
MFKKYSSLENHYNSKFIEKLYTNGLTTGVWVAREKIHGTNFSLIIERDNVTCAKRTGPILPAEDFYGYEIVLKKYDKAIKAVQEVMESISTSVPVSYQVFGEFAGGGIQKGVDYGEKDFYVFDIIINTESDDTYYMSDYEMQDFCNTFGFKMAPMLGRGTFDSLIMIPNDLDSVLAAYNSTASEDLVEANNCVFDANVIGDNTAEGYVLKPCFPKWLSNGTRVAIKCKNSKFSEKKKSDKPVKTQVPLTEIDKNLLDVLACYVTLNRVNNVISKIGTVTPKDFGKVMGLTVQDILEETSREGIVLTSSDNPNLVKKELVRMVQDVLRPAWIELVS

SEQ ID NO: 11 - protein, 372 aa, Bacteriophage RB69
MEKLYYNLLSLCKSSSDRKFFYSDDVSPIGKKYRIFSYNFASYSDWLLPDALECRGIMFEMDGETPLRIASRPMEKFFNLNENPFTLSIDLNDVKYLMTKEDGSLVSTYLDGNMVRFKGSIKSDQAASATSILLDINHKDLADRLLELCNDGFTANFEYVAPSNKIVLTYPEKRLILLNIRDNNTGKYIEYDDIYLDPVFRKYLVDRFEAPEGDWVPGVKSSTNIEGYVAVMKDGSHFKLKTDWYVALHTTRDSISSPEKLFLAIMNGASDDLKAMYADDEFSFKKVELFEKAYLDFLDRSFYICLDAYDKHKGKDRKTYAIEAQAICKGAQSPWLFGIIMNLYQGGSKEQMMTALESVFIKNHKNFIPEGY

SEQ ID NO: 12 - protein, 269 aa, Aeromonas virus Aeh1
MIVGRYEKQIRQLHKCLVHLDMIDKEDSIGVFGEYAGIMSYGKWIQTGIEYGPQDFYVFDIIVQPLDGDQFMLEDLQVEELCKALGLKTAPLLKVGTFADIMKIPVDLQSVVMEVNAGKPIDIRVGTDNIAEGYVAKPNVPARFKNGNRVAIKCKNEKWSETGKGRAVQVEVKELSEKDKALVLDITRYITDNRLKNVLSKMDTPKTSEFGKVLGLMSKDVQKDYERDELDGVSVKEATDEAGRVMRMINTEIGNMIRPNWVSICDGDW

SEQ ID NO: 13 - protein, 334 aa, Vibrio phage JS98
MFKKYSSLENHYNSKFIEKLRTNGLTGGEWVAREKIHGTNFSLIIERDAVTCAKRTGPILPAEDFYGYEIVLKNYADSIKSVQHLIESINYQSYQIYGELAGPGIQKNVDYGDKDFYVFDIRVTKEDGTESVLTDTLMEAFCIIHKFKVAPCLATGSFEDLIKLPNDFDSVIPDYNFAVDNAGLTIANSTDFIPKVEGKVFTAEGFVLKPDIPTWLPNGNRVAIKCKNSKFSEKKKSDKPIKAAVVLSQDDMDLMWQFTDYVTVNRINNVISKIGEVSKKDFGKVMGLTVQDILEEAAREELELTDAENPVEVKKQLVECVKDTLRAVWIELVS

SEQ ID NO: 14 - protein, 335 aa, Vibrio phage
MSFVKYTSLENSYRQAFVDKCDMLGVREWVALEKIHGANFSFIVEFKPNEAQDGAEFTVTPAKRTSTIGANVMGDYDFYGCTSVVEAHTAKMEAISNWLWARGIINVGETIIVYGELAGKGVQKEVNYGDKDFWAYDILLPETGKFLDWDVVLEACEFAKVKTTHEIARGTLDELLRIDPLFRSFHTPADVDGDNVAEGFVVKQLRNEKRLHNGSRAILKVKNDKFKEKKNKAGKTPRAAVVLTEEQEKLHAAFSCYLTENRLRNVLSKLETVTQKQFGMISGLFIKDAKDEFERDELNETAIARDDWDVIKRSLTNIANEILRKNWLDILDGNF

SEQ ID NO: 15 - protein, 382 aa, Acidobacteriabacterium
MKQMYDNLKALTQKNDMFFSSIQTTPSNKPVEIFSYHIASYSDWLEPDAIECRGIMFDITDKENPVILSRPMEKFFNLGENPLALPEDVLPLVKTIEEKRDGSLISTYLDDGKLYTKSKGSLYSDQANDSNRFLMRSENKDFKQALKTLAELGYTANMEYTSPKNQIVLKYEKQELIVLNIRNTETGDYLTLDDLAELDAENPEHTIYTHIAERFVDYEEVDGMSDEDVERIRDMKGIEGYVLVGQNQRVKLKTDWYVNLHRLKDNINNNRRLVESVVESRTDDLRQLFEHDQGSIDKIKEFEQYVLSKIKSCLAEVRTVYERVKHLDRKHYAINAQRYVDYTPLFSVIMRQFDDYNEENVVENIKQIALKNVDDFIPMHYK

SEQ ID NO: 16 - protein, 379 aa, Vibrio phage nt-1 rnlA
MNELYNNLMTLAESAEGKFFFADHLSPQGEKFRVFSYHIASYSDWLLPDALEARGIMFQLDENDEMIRIVSRPMEKFFNLGENPFTMDLDLTTTVQLMDKADGSLISTYLTGDNFALKSKTSIYSEQAVAANRYIKHVDNRDLWEFCDDCAAQNFTVNMEWCAPNNRIVLEYTEPKLIILNIRDNETGQYVSFDDIPIGALTRIKKWLVDEYDPMTAHVDDFVETLKAKKGIEGMILRLASGQSVKIKTTWYVDLHAQKDSVNSPKKLVTTILNKNHDDLYALFADDKPTIERIREFDDHVSKKVVESFHAVSQYYTKNRHLSRKDFAIAGQKALKPWEFGVAMIAYQNQTVEGVVTMLINAYLKRPELLIPEKYLSEV

SEQ ID NO: 17 - protein, 351 aa, Streptomyces phage Wakanda
MVHVSEIFSTDDLEQAIENGYVRVNPHPTAPLAILGYTEKAQFDRMWNDVTLNCRGLIIDHDGFVVARPWKKFFNFGERPLMFDTDAPVEVTDKKDGSLGILYRDPVTGDYAISTRGSFTSDQAIHATELFNKKYSHIVTPFKETTFLFEIVYPKNRIVLNYGDMDDLILLGAVDNERGYYWGPRQAAGIMGWPGPVTEVFRYRSLNECFGVHRENAEGLVIRSGSDMVKLKQADYVELHRIVTNLNERSVWSQLKDGKAAYQICELIPDEWHEWVVDVAQALWTEYSSLENKVLGTYADLIGELPGGFTRKQFAMKATKTPYAGYLFALLDCKSISDMLWEAVKPEVNNK

SEQ ID NO: 18 - protein, 331 aa, Morganella phage vB_MmoM_MP1
MFKKYNSIENIDNAKLVDKVRYEGFTDPSVQWIAQEKIHGANFSFMYDGKTLKCAKRSGDIKETESFFGYEIILAQYKKSVLDAWDILVEHFKGVEEINIFGEFAGPGIQKEVDYEHKDFYAFDILVNGRYIDKEIVNETCKLARIKLAPIIRYGSFDELCNMERAFDTLVPKYNEMLKKNTDAFDFIFGEQEEGKDNISEGYVISPVVPAHLTNGNRVIFKCKNAKFKEKGKIREVKPVKELSESDMKFVELATAYITEQRLSNVISHIGEIGPKDFGKVMGLMSKDVYEDMAKDGFDVLETTDIPLVKKTIQMEITTFIRKDWVNYVSR

SEQ ID NO: 19 - protein, 336 aa, Flavobacterium terrae
MEFRKYNSIENTYQKTVLEQIIKHEFDAVEYVVQEKVHGANFAFYTNDIQVKIAKRSDFIEENDTFYNAHKVAQKYHAKVKSLFYEVKELFPNVQFIAVFGELFGGHYNHPEVPTVQGAIKVQKGIHYSPENDFYAFDIKVDNSHYLNVDLANKLFEKTDFFYAKTLFKGSLADCLKYPNDFNSLIPEWLDLPTLETNIVEGVIIRPVEALFFGNGSRVLLKNKNEKWAEKAKCDKSKKDLALVDFPIEAKPVWSKIKDYVTVNRLYNVLSKEGEFYPKIIGKLTGWMSQDVINDFKKENPSELDTLEKESQRAINKRLNTMVIKLIKEEFMTFEV

SEQ ID NO: 20 - protein, 332 aa, Klebsiella phage vB_Kpn_F48
MFEKYSSLENHYNNRFIEKIRHHGYDVTEGWCAREKIHGTNFSIIIERDAVTCAKRTGPILPAEDFFGYTVILKKYNDSIKAVQHTIKEGSSMQIFGEFAGSGIQKGVDYGEKDFYVFDILVKTDKGTHQFVDDFMMEQMCCTFGFKVAPLMGRGSFDELAKLPNEFQINVNRYNEAAEVDLRNANTRVWPAEEATDNTAEGYVLKPNYPRFLANGSRVAIKCKNSKFSEKAKSDKPIKPKAVLSEIDQEVLQKFSEYVTIQRVNNVISKIGQVGPKDFGKVMGLTVQDILVEAGREGLEVIQAEQPDIVKKEITKLVQDVLRPAWIELVSN

SEQ ID NO: 21 - protein, 334 aa, Escherichia phage EcS1
MTFEKYSSLENHYNGKFIEKIRFSGNDTGVWVAREKIHGTNFSLIISRDAVTPCKRTGPILPGESFFAHEIIMKKYDKSIKFLQDSICGTASSYQIFGEFAGGGIQKGMDYGEKDFYVFDILIKSEHDQEGTYADDFMVERMCCTFGFKVAPLIARGSFEELSQLVNDFDSVVNHYNELAVANGIEYANIAHFGFLPHGEKNIAEGYVLKPCYPVILANGNRVAIKCKNSKFSEKAKSDKPIKPAAVLSDQDKVALSTLAEYSTWNRVSNVLSHIGEVTAKDFGKVMGLTMQDIFVEAEREGIVLIDADQPNLVKKELQQIVMATIREKWHEVV

SEQ ID NO: 22 - protein, 340 aa, Acinetobacter phage AbTZA1
MSFIKYSSLENHTNDKFIQKCFEAVANGEGTVNTEFVAREKIHGTNFSVIITPDSIQAAKRSGPIAITEKFFGYEDLMAELDDIFKEIQQDLVKNVPSFKSIQIFGEYAGGGIQKEVDYGPKSFYVFDIFMDAPDSGFSHGWWSDVNVQAFCDYRGLKIAPLVARGTLEQLLKLPVEFDSIVPSLTWENMYSVHAQPAPKDNVAEGLVIKPNSPMFLPNGSRLAIKYKTDKFKEKGKGKAPKIPVPLSDADKELLNKLSEFSTIARISNVASHIGELTPKMFGKLLGMTMHDLLTEAEREGISPKSAEAPSKVKNELQKIVQVDVREFWTSYDFPVVNVD

SEQ ID NO: 23 - protein, 335 aa, Klebsiella phage KMI11
MFAKYSSLENHYNNKFIEKIRGAGFDMHTVEWVAREKIHGTNFSVIITPTEIVPAKRTGPILESESFFGHDIIMKKYKDSFVKMQNMLNAMDLVSVQIFGEFAGGGIQKGVDYGEKDFYVFDILSDSGNEKVYWDDYVVESFATGLGLKLAPLLGRGSFAELSQYVNDFKSIVNYYNELVDTTDLEHANKHVFGPQASSETGVAEGYVLKPVHPKFFNNGTRVAIKCKNSKFSEKAKSDKPIKAKVELTENDKRVLEIFSEYVTWNRVSNVLSHIGTVTAKDFGRVMGLTMKDIINEAAREGHDMLFADNPSAVKKEITTLIQNTIRSKWHEVLE

SEQ ID NO: 24 - protein, 366 aa, Yasminevirus sp. GU-2018
MSTPPFLKYSSIESYTDVKHLEKIRQIFKSDQFTASEKVHGANFQFIVNEDASNNKISIACAKRTSILEDSEEFYDWRNVLSKHRASLEILYQKVKTDLNKYTGDSSTKNLAGVRVYGELFGGEYPGHGKKNLKPVQKWIYYNTDIDFIVFDVVVVINSDSPDHTSETFLSSDDVMDLICSCSSLKSDDDSVFSLKTVPILSRGSLDEVIEFCTKNVQFNTKIPHLYGLPDIENNFAEGYVVKANVRVNVGKHRGVVKVKNPKFDEIIGFVRHDKRDKKSTNDVSEEVKYHTEMIKPYLTQNRLDNVVSKIGPASVRPKIVGCFLNDAKIDYIKSFDDDDSVKDFEKVWKDVQKNLTPLCNTFVYP

SEQ ID NO: 25 - protein, 334 aa, Enterobacter phage vB_EclM_CIP9
MFEKYSSLENHYNGKFIEKIRNAGFDVTEPWVAREKIHGTNFSIIIERDAVTCAKRTGPILAGEDFFGYEIVLKKYNDSIKAVQHTIKEGSSMQVFGEFAGGGIQKGVDYGEKDFYVFDILVKTAEGTNQFVDDYMMETICNTFGFKMAPLLGRGKFDDLIQLPNMLDVVVNDYNELAANEGIPVANKQVWKAVVAEDNIAEGYVLKPCYPKFFPNGSRVAIKCKNSKFSEKSKSDKPIKPKVELTEQDNKVYFDFESYINVNRINNVVSKIGKPGPKDFGKVMGLTVKDLLEEAEREGIVLTTADNPDLVKKAIIKTTQDVLRHVWQYLISDE

SEQ ID NO: 26 - protein, 335 aa, Escherichia phage CJ20
MFKKYNSLENHYNNKFIEKIRLQGFTSGEWVAREKIHGTNFSLIIEQDNVTCAKRTGPILPAEDFYGYEIVLKNYADSIKSVQKLLQDINYQAYQIYGEFAGAGIQKNVDYGDKDFYVFDIRVTKEDGSESVLTDTLMEAFCIIHKFKVAPRLATGSFEDLIKLPNDLDSVVPDYNFTVDNAGLTTANTTDFDAKVEGKVFTAEGFVLKPDVPAWLPNGERVAIKCKNSKFSEKKKSDKPIKAAVVLSQEDLDILWKFTDYVTVNRINNVISKIGEVSPKDFGKVMGLTVQDILEEAGREGLELTQSENPVEVKKQLITNVRETLRHVWIALISE

SEQ ID NO: 27 - protein, 322 aa, Cronobacter phage A24
MKFEKFQSLINESMKNVGGFLRDSSFGKRKAVVTEKIHGANFSVYFGCKDNVVGINFASRSQMLCPETNFMNCQRYFTEEKIQELLEHASTIMALDKCELRFIGEIYGGMDIAGIKPVQREVHYSGDIGFRVFHAQIANNETGEVFDYNWKNVKALASDFGFEVVPIVAEGLTFEQAYALDQKVKSALSDKDQICEGYCIRVDADGEEGQAPLIFKKRNTDFLETKGTVKAPQNTVEQTELGMEAMARIGSFITPQRVSNVNSHHGYSSPKDFQNLMAAVLEDVLDEYKKEYDVDLRNEPVWKEIKRSVGAQVVPLVREVLL

SEQ ID NO: 28 - protein, 352 aa, Rotaria sp. Silwood1
MSEFEGYGKISESSSNWTLEKSDNTTFKRILWCVTEKVHGANFCFLCDNNGQRIQCGKRTSLLSDTDEFFGYKRRLFNEIIPKIQQIYQFVQNTFPNLEKLYVFGELFGGYYPHPDVPKLPNINAIQTGIWYCPDIEFYAFDLAISINDKQTYLDYEYAITAFQHVNLLYAEPLFIGKYEEALDFKLGFNSHIPGKLGLPPLHEDNKAEGIVIKPMHEIMIKTNKGSPIRAIVKKKIEEFAEDKYNQAQKQVFKNDEQFSNVDLLRFEIDALITDNRLNNALSKVGHVTRDDKEKLKELLNIYVKDIMDQLYENGNEDMWNNLSSNDRNLFTEELTLNAKKVILKYLKTNKC

SEQ ID NO: 29 - protein, 346 aa, Acinetobacter phage Ac42
MPFVKYSSLENHTNSKFLEKIVEAITLGYCDNHFVAREKIHGTNFSVIITKDSIQPAKRSGPISETESFFGWQDLMAKYRKSFEVIQEKLIAGEYKQEIEGSPGFVPSVTVEKVQIFGEYAGGGIQKEVDYGEKDFYAFDVMFDDKYINDVAATGVASVAGLKMAPIIAIGTLEELLKLPVEFNTTVPTYNKLWDEAGNGFYDFVKPEAPTDNVGEGLVIKPVVPAFLGNGSRIAIKYKTDAFKEKGKGKAPKLPTPMTDKDIALATQFSEFITENRLSNVLSHIGEVTAKDFGKVMGLMMKDIFAEAKREEISIDVADSPSKVSKEIQHQVTTLIRSKWVDIISN

SEQ ID NO: 30 - protein, 307 aa, Helcococcus kunzii ATCC 51366
MKFTRYPSLTNHYAIGKTRDLIGKLDDEYYATEKNHGTNIQLTVDKNLRVGVGKRSTFITDEKPYSDVFELSEDIIAELQGFIAENADIEQVTLYGELFGSGVQKTDYQANKDKERQVRFYDCFIHFTNGKIIASKKDLYELVKEEFVAKIIKTGKLIDLVKEELPKESTYGGNTFEGYVYKPNVDNYVLNSNNNGIYYPVVKHKTEDFSEVRNKVKIELGEEEIKLHNLVESYITKNRVVNVLSHGDIELIPQNIGEIIKLVQEDIKKELIKENPEVDKNLVYQIVRKKGSLIVPLIKKIMFEEVE

SEQ ID NO: 31 - protein, 382 aa, Vibrio phage CHOED
MLRPFEKYNSLTLIRENHEDELQKYIDLTQGQRFVVTEKIHGANFEVATDGQTVRYASRNQVLGEGADFYGYRFVAQFLTPKILAMFKDMKELIMEQHKACDYIEAKGDQANRPDIPRDFQEITIRGELAGGQYPNAPKVKEGNGQVGKGKIWYSQQKSFFAFEICVDGVPQDFYTLGTMCGSYGIPVAPVLTFGTFEECLEFSREHLEDITTVPNMTPLLNENGHPILNEDSSYCALHPIHNNTREGHVISSVNPVYLPNGKRMVFKHKGVKFMENKGEKKPKAKVEVILTPEQQVVFDTILPMITVARMEAVMSKEGTWEPKDFTKLCGKVLEDATDEAHGDAPNAFFAAWAHISTKERKVVMKQLGREAAERLRTAYFS

SEQ ID NO: 32 - protein, 334 aa, Cronobacter phage S13
MFKKYNSLTNHTDKKFLNKILFAGLTDPKVLWVAREKIHGANFSFIVTSDSVSVGKRSGVIPEGENFYSHADIESRYRADVISVRRRLIDLGIATETSEIQIYGELAGVTSTGKLIQHGVDYGPSDFYVFDITVDGVYQDDTTCVLALTRTNITMAPFLKMGTFDELISMRNDFDSVVQRWKNDFNAIVWDKGEHLQYTETNTAEGFVMKPTEVHYVGMERVAIKHKNEKFSEKKNKVKNFKAPVPMTEKDQEVLDELLTFNTENRVRNVLSKTGTPDTKQFGMIMGLTVKDILEESKNILDTADAPATVKKTLIAEVSNLIRPHWVNICNGEF

SEQ ID NO: 33 - protein, 271 aa, Thecamonas trahens ATCC 50062
MEGMVEAVAAAFVPYPKIPTAFSGSADDARRVRTIEWVATEKIHGANLTLMCDGQVVVPAKRRGVLADDEDFFGLRSSGLLASLARPAIELAQALGAGSGTSIAVSGELFGADVQPGIDYGPQLQFAVFDVALLAADGDRRFLAHDEMTAVATAAGFTVVHEVARGSYTKLLDTPIGFDSHWPALLGLEPLPPAGANTAEGIVLRPATTDDRFLVKIKDPSFADVEASGRAHKSMMVAADGSSSAAADAQNIFYELQLYLTPARAQSARDW

SEQ ID NO: 34 - protein, 367 aa, Acinetobacter phage vB_AbaM_phiAbaA1
MMKFIKYPSIKRLTERAIHELDKLPFDLPVFVVTEKLHGANMGIYCDGETIRIAKREGFQDECETKNFFDSARVAEKYSESILGLVRSWNLVKKSHGLEGYAYYIFLGELFGGGIHKGTPYSMEQDFALFNIFTVIDDTEANREYVKKLCAAYFEDEVNGKLVLMPQSRERIVNIAKYINCKVLDILFKGTLEECAQFANDFESHFVCPNRVRESGVEKHGDDAVKNLCITEGVIIEPFYYTNYKGNNFTYKSKNAKFEEKYATGYKPKVSLVQKAIDNLTEDQAEMLYTLNEYLVMPRYQSVVSKMGEVTIKDFSKVLKAFVEDVLKDAKEDFAEDGKEFVKPTKDMMMLFTNEVKSYIRPILLGE

SEQ ID NO: 35 - protein, 335 aa, Klebsiella phage Mineola
MFAKYSSLENHYNGKFIEKIRGAGFDMHTVEWVAREKIHGTNFSVIITPTEIVPAKRTGPILESESFFGHDIIMKKYKDSFVKMQNMLNAMDLVSVQIFGEFAGGGIQKGVDYGEKDFYVFDILSDSGNEKVYWDDYVVESFATGLGLKLAPLLGRGSFAELSQYVNDFKSIVNYYNELVDTTDLEHANKHVFGPQASSETGVAEGYVLKPVHPKFFNNGTRVAIKCKNSKFSEKAKSDKPIKAKVELTENDKRVLEIFSEYVTWNRVSNVLSHIGTVTAKDFGRVMGLTMKDIINEAAREGHDMLFADNPSAVKKEITTLIQNTIRSKWHEVLE

SEQ ID NO: 36 - protein, 327 aa, Enterococcus phage 9181
MPFFKYPSLTNEYAVAKSRSILSKMNTIAYSTEKIHGSNVQYVFDDRDDVVNFGAFSRNGKKVGGKDDNGEHIVDTQFKLVMDIAFQMDLPNIASSIFTEFNHVDSINIYGEYFGSGVQRTQYFINERNERGFQVFDIFLHYKGDPQEVYRSMGLLELIDFVGRDKMVPIEDIVFLSNLIEKDIVERSHYGGEREGNVYKEIHGSWIDPVTKYCGIKHKRPEFLEVSKAPKQPKAKLSDEFLEVVERLSTYVTENRVRNIHSHGDIKFITKNIGAIMLEVKKDILKEFEDNEESIPNVDLSKAIRACDRDIALAVRKVIAEVGDMED

SEQ ID NO: 37 - protein, 329 aa, Aeromonas phage Ahp1_CNU-2021
MIFKSYPEMENHSKSRIINAVIEQGHGAADVVWCAREKIHGTNFSLWYNGVDDVRAARRTDFLEFADKFYDFTNIERRYQLCVQALYLRLGLTTEVMAVYGEYAGIMSSGKWIQTGIEYGPQDFYAFDVMVDGVPIDDDVMESACLDCGMKTAPLLKVGTFKEVMGVPNDLQSVVMTKNETGTFEIVKGTDNIAEGYVAKPRVGRRFWNGARVAIKCKNEKWSETAKGKGVKIEVKDISDKDASILAMLGDYITENRLKNVLSKIGVPETKEFGKVMGMLSQDIIKDYESDTETLVKDADEPSRVCRMMNTAVGNFIRPLWVDICDGAW

SEQ ID NO: 38 - protein, 382 aa, Megavirus chiliensis
MIIFWKDTYIYYDIIKNLKKNNIECTDYIIYIITTMNMEINQFFQKYFSIENLNARSFKSLQKNGLLSNNIEWIALEKIHGANFSFITNGEKLETAKRTGIISSEEYFFNYQIVVERYSQDVFNIFNKIKKNIDNLMSIQIYGELFGGAYPDMYVKDIKPIQKGVYYNPDIDFLIFDIKINYKTESGIPENNYSEFLSHDEVINYISKTNIRIVPEISRAIFTDIIKMDPVFHTKVPAMYGLPQINNNLAEGYVFKMNARHLCNIFRPIIKSKNDDIFGEVHKSSIKYDIKDLLLKNSEIGSSYEEIKCYLTKNRFDGIIGKIGPDNKPAKIIGCFIADALREYEITLDADKKIEYNKNKRNISKNITIYISNNPEIQSWFK

SEQ ID NO: 39 - protein, 218 aa, Acanthamoeba polyphaga moumouvirus
MELAKNFQKYFSIENPKKIIKSLEKNDYTNDKYEWIVLEKIHGANFSFITNGETIYAAKRTAIIQPGEYFYDYESIVEKYKEDVFKVYNEIFYKTKNIMSIQIFGELFGGLYPNYNDKKINPIQTGIYYNPKIDFMVFDIKINYLTDNFNVQNDKSEFLSHDEVLFYLSTTKFKHVPIIGRGQFNDIIKMEPVFLLKYLEYMNYLMLIIIMLKGIYLN

SEQ ID NO: 40 - protein, 335 aa, Salmonella phage S16
MFKKYSSLENHYNNKFISKIRFEGKDGGLWVAREKIHGTNFSIIVSKDSVSACKRSGPILPSESFYGHEIILKNYDESIKTIQRCMNANELGSVSSYQIFGEFAGQGIQKEVDYGEKDFYVFDILVNTQNGNVLYMDDMMMTSFCNEFGFKMAPFIGCGSFDELIQLPNNFTSVIKAYNEAAKDDLKEVNLCVFDPLVTDDNVAEGYVLKPVYPDFFNNGTRIAIKSKNSRFTEKKKSDKPIKPKAVLTSNDSTVLANLCEYSTWNRVSNVISHIGEVKAKDFGKVMGLTIQDIFIEAKREGVDIVHADNPDLVKRELQTVVSNTIREKWLEIVS

SEQ ID NO: 41 - RNA, 14 nt, synthetic construct
  source 1..14: mol_type = other RNA; note; note (original language) = 底物1
  modified_base 11: mod_base = OTHER; note = Thymine; note (original language) = 胸腺嘧啶
ctagacctgttttg

SEQ ID NO: 42 - skipped

SEQ ID NO: 43 - RNA, 10 nt, synthetic construct
  source 1..10: mol_type = other RNA; note; note (original language) = 底物3
aggtctagaa

SEQ ID NO: 44 - RNA, 13 nt, synthetic construct
  source 1..13: mol_type = other RNA; note; note (original language) = 底物4
acaaaagcaaaac

SEQ ID NO: 45 - RNA, 21 nt, synthetic construct
  source 1..21: mol_type = other RNA; note; note (original language) = 正义链
  modified_base 11: mod_base = OTHER; note = Thymine; note (original language) = 胸腺嘧啶
ctagacctgttttgcttttgt

SEQ ID NO: 46 - RNA, 23 nt, synthetic construct
  source 1..23: mol_type = other RNA; note; note (original language) = 反义链
acaaaagcaaaacaggtctagaa

SEQ ID NO: 47-53 - skipped (7 entries)

SEQ ID NO: 54 - RNA, 13 nt, synthetic construct
  source 1..13: mol_type = other RNA; note; note (original language) = 底物12
  modified_base 3: mod_base = OTHER; note = Thymine; note (original language) = 胸腺嘧啶
gttttgcttttgt

SEQ ID NO: 55 - RNA, 15 nt, synthetic construct
  source 1..15: mol_type = other RNA; note; note (original language) = 底物13
aaaacaggtctagaa

SEQ ID NO: 56 - skipped